European Patent Application EP 4 365 197 A1, published May 8, 2024. Title: Humanized antibody specific for CD47 and a pharmaceutical composition for preventing or treating CD47-related diseases comprising the same. Applicant: InnoBation Bio Co., Ltd. The sequence listing filed with the application follows.

SEQUENCE LISTING (123 sequences)

SEQ ID NO: 1 - protein, 8 aa, Artificial Sequence
  3A5 VH_CDR1
GYTFTSYW

SEQ ID NO: 2 - protein, 8 aa, Artificial Sequence
  3A5 VH_CDR2
IDPSDSYT

SEQ ID NO: 3 - protein, 10 aa, Artificial Sequence
  3A5 VH_CDR3
ARGGKRAMDY

SEQ ID NO: 4 - protein, 11 aa, Artificial Sequence
  3A5 VL_CDR1
QSLVHSNGNTY

SEQ ID NO: 5 - protein, 3 aa, Artificial Sequence
  3A5 VL_CDR2
KVS

SEQ ID NO: 6 - protein, 9 aa, Artificial Sequence
  3A5 VL_CDR3
SQSTHVPFT

SEQ ID NO: 7 - protein, 117 aa, Artificial Sequence
  3A5 VH amino acid sequence
EVQLQQPGAELVKPGASVKMSCKASGYTFTSYWMHWMNQRPGQGLEWIGVIDPSDSYTSYNQKFKGKATLTVDTSSSTAYMQLSSLTSEDSAVYYCARGGKRAMDYWGQGTSVTVSS

SEQ ID NO: 8 - protein, 112 aa, Artificial Sequence
  3A5 VL amino acid sequence
DVLMTQTPLSLPVSLGDQASISCRSSQSLVHSNGNTYLHWYLQKPGQSPKLLIYKVSNRFSGVPDRFSGSGSGTDFTLKISRVEAEDLGVYFCSQSTHVPFTFGSGTKLEIK

SEQ ID NO: 9 - DNA, 351 bp, Artificial Sequence
  3A5 VH nucleotide sequence
gaggtccagctgcagcagcctggggctgagctggtgaagcctggggcttcagtgaagatgtcctgcaaggcttctggctacaccttcaccagctactggatgcactggatgaaccagaggcctggacaaggccttgagtggatcggagtgattgatccttctgatagttatactagctacaatcaaaagttcaagggcaaggccacattgactgtagacacatcctccagcacagcctacatgcagctcagcagcctgacatctgaggactctgcggtctattactgtgcaagagggggtaagagagctatggactactggggtcaaggaacctcagtcaccgtctcctca

SEQ ID NO: 10 - DNA, 336 bp, Artificial Sequence
  3A5 VL nucleotide sequence
gatgttttgatgacccaaactccactctccctgcctgtcagtcttggagatcaagcctccatctcttgcagatctagtcagagccttgtacacagtaatggaaacacctatttacattggtacctgcagaagccaggccagtctccaaagctcctgatctacaaagtttccaaccgattttctggggtcccagacaggttcagtggcagtggatcagggacagatttcacactcaagatcagcagagtggaggctgaggatctgggagtttatttctgctctcaaagtacacatgttccattcacgttcggctcggggacaaagttggaaataaaa

SEQ ID NO: 11 - protein, 117 aa, Artificial Sequence
  Hu3A5(V1) VH amino acid sequence
EVQLVQSGAEVKKPGASVKVSCKASGYTFTSYWMHWMRQAPGQGLEWIGVIDPSDSYTSYNQKFQGRVTLTVDTSTSTAYMELSSLRSEDTAVYYCARGGKRAMDYWGQGTTVTVSS

SEQ ID NO: 12 - protein, 112 aa, Artificial Sequence
  Hu3A5(V1) VL amino acid sequence
DVVMTQSPLSLPVTLGQPASISCRSSQSLVHSNGNTYLHWFQQRPGQSPRLLIYKVSNRFSGVPDRFSGSGSGTDFTLKISRVEAEDVGVYFCSQSTHVPFTFGGGTKLEIK

SEQ ID NO: 13 - DNA, 351 bp, Artificial Sequence
  Hu3A5(V1) VH nucleotide sequence
gaggtgcagctggtgcagagcggcgcggaggtgaagaagcctggtgctagcgtgaaagtttcctgtaaagcgtctggctacacgttcacaagctattggatgcactggatgcgccaggcccccggccagggcttggagtggatcggtgtgattgacccgtccgacagctacaccagctacaaccagaagttccagggtcgtgtcaccctcactgtggacacctcgacctccaccgcctacatggagctgagctccctacggtctgaagatacagccgtgtactactgtgctcgtggtggcaagcgcgccatggattattggggccagggcaccaccgtcactgtatcgtcc

SEQ ID NO: 14 - DNA, 336 bp, Artificial Sequence
  Hu3A5(V1) VL nucleotide sequence
gatgtggtgatgacccagtctcctctttccctgcccgtaaccctcggacagccagcatctatctcatgccgatcctcccagagccttgtccactcaaatggcaacacgtacctgcattggttccagcagaggcctgggcagagcccgcgcctgctgatctacaaggtgagtaaccgcttttctggggtgcccgaccgcttcagtgggtcgggctccgggaccgactttactctgaagatttcccgcgtggaggccgaggacgtgggcgtctacttctgctctcaatctactcacgttcccttcaccttcggcggcggtaccaagctggagatcaag

SEQ ID NO: 15 - protein, 244 aa, Artificial Sequence
  Hu3A5(V1) scFv amino acid sequence
DVVMTQSPLSLPVTLGQPASISCRSSQSLVHSNGNTYLHWFQQRPGQSPRLLIYKVSNRFSGVPDRFSGSGSGTDFTLKISRVEAEDVGVYFCSQSTHVPFTFGGGTKLEIKGGGGSGGGGSGGGGSEVQLVQSGAEVKKPGASVKVSCKASGYTFTSYWMHWMRQAPGQGLEWIGVIDPSDSYTSYNQKFQGRVTLTVDTSTSTAYMELSSLRSEDTAVYYCARGGKRAMDYWGQGTTVTVSS

SEQ ID NO: 16 - DNA, 732 bp, Artificial Sequence
  Hu3A5(V1) scFv nucleotide sequence
gatgtggtgatgacccagtctcctctttccctgcccgtaaccctcggacagccagcatctatctcatgccgatcctcccagagccttgtccactcaaatggcaacacgtacctgcattggttccagcagaggcctgggcagagcccgcgcctgctgatctacaaggtgagtaaccgcttttctggggtgcccgaccgcttcagtgggtcgggctccgggaccgactttactctgaagatttcccgcgtggaggccgaggacgtgggcgtctacttctgctctcaatctactcacgttcccttcaccttcggcggcggtaccaagctggagatcaagggcggcggaggctccggtggaggcgggtccgggggaggcggctcggaggtgcagctggtgcagagcggcgcggaggtgaagaagcctggtgctagcgtgaaagtttcctgtaaagcgtctggctacacgttcacaagctattggatgcactggatgcgccaggcccccggccagggcttggagtggatcggtgtgattgacccgtccgacagctacaccagctacaaccagaagttccagggtcgtgtcaccctcactgtggacacctcgacctccaccgcctacatggagctgagctccctacggtctgaagatacagccgtgtactactgtgctcgtggtggcaagcgcgccatggattattggggccagggcaccaccgtcactgtatcgtcc

SEQ ID NO: 17 - protein, 117 aa, Artificial Sequence; identical to SEQ ID NO: 11
  Hu3A5(V2) VH amino acid sequence

SEQ ID NO: 18 - protein, 112 aa, Artificial Sequence
  Hu3A5(V2) VL amino acid sequence
DVVMTQSPLSLPVTLGQPASISCRSSQSLVHSNGNTYLHWFQQRPGQSPRLLIYKVSNRFSGVPDRFSGSGSGTDFTLKISRVEAEDVGVYYCSQSTHVPFTFGGGTKLEIK

SEQ ID NO: 19 - DNA, 351 bp, Artificial Sequence
  Hu3A5(V2) VH nucleotide sequence
gaggtgcagctggtgcagtctggtgcagaggtgaagaagcctggtgcttccgtgaaagtatcttgtaaggcttctggctacacgttcaccagctattggatgcactggatgcgccaggcccccggccagggtttggagtggatcggtgtgattgacccgtccgacagctacacctcctacaaccagaaatttcagggccgcgtcactcttaccgtggataccagcacttcgaccgcctacatggagctgtcctctctgcgcagcgaggacaccgcggtgtactactgcgcccgtggcggcaagcgcgccatggattattggggccagggcactaccgtcacagtgtccagc

SEQ ID NO: 20 - DNA, 336 bp, Artificial Sequence
  Hu3A5(V2) VL nucleotide sequence
gacgtggtgatgacccagagtccactttcgctgcctgtcacactaggacagccggcgtccatctcgtgccgatcgtcccaaagcctcgtccactcaaatggcaacacgtacctgcattggttccagcagcgccccgggcagagcccacgtctcctgatctacaaggtgagtaaccgcttctctggcgttcccgacaggttttcaggatctgggtccggcaccgacttcaccctgaagatctctcgggtggaggctgaagatgtgggcgtttattactgttcgcagagcactcacgtccccttcaccttcggcggggggaccaagctggagatcaag

SEQ ID NO: 21 - protein, 244 aa, Artificial Sequence
  Hu3A5(V2) scFv amino acid sequence
DVVMTQSPLSLPVTLGQPASISCRSSQSLVHSNGNTYLHWFQQRPGQSPRLLIYKVSNRFSGVPDRFSGSGSGTDFTLKISRVEAEDVGVYYCSQSTHVPFTFGGGTKLEIKGGGGSGGGGSGGGGSEVQLVQSGAEVKKPGASVKVSCKASGYTFTSYWMHWMRQAPGQGLEWIGVIDPSDSYTSYNQKFQGRVTLTVDTSTSTAYMELSSLRSEDTAVYYCARGGKRAMDYWGQGTTVTVSS

SEQ ID NO: 22 - DNA, 732 bp, Artificial Sequence
  Hu3A5(V2) scFv nucleotide sequence
gacgtggtgatgacccagagtccactttcgctgcctgtcacactaggacagccggcgtccatctcgtgccgatcgtcccaaagcctcgtccactcaaatggcaacacgtacctgcattggttccagcagcgccccgggcagagcccacgtctcctgatctacaaggtgagtaaccgcttctctggcgttcccgacaggttttcaggatctgggtccggcaccgacttcaccctgaagatctctcgggtggaggctgaagatgtgggcgtttattactgttcgcagagcactcacgtccccttcaccttcggcggggggaccaagctggagatcaagggcgggggaggctccggcggaggcggctccggtggtggtggctccgaggtgcagctggtgcagtctggtgcagaggtgaagaagcctggtgcttccgtgaaagtatcttgtaaggcttctggctacacgttcaccagctattggatgcactggatgcgccaggcccccggccagggtttggagtggatcggtgtgattgacccgtccgacagctacacctcctacaaccagaaatttcagggccgcgtcactcttaccgtggataccagcacttcgaccgcctacatggagctgtcctctctgcgcagcgaggacaccgcggtgtactactgcgcccgtggcggcaagcgcgccatggattattggggccagggcactaccgtcacagtgtccagc

SEQ ID NO: 23 - protein, 117 aa, Artificial Sequence; identical to SEQ ID NO: 11
  Hu3A5(V3) VH amino acid sequence

SEQ ID NO: 24 - protein, 112 aa, Artificial Sequence
  Hu3A5(V3) VL amino acid sequence
DVVMTQSPDSLAVSLGERATINCKSSQSLVHSNGNTYLHWYQQKPGQPPKLLIYKVSNRFSGVPDRFSGSGSGTDFTLTISSLQAEDVAVYFCSQSTHVPFTFGGGTKLEIK

SEQ ID NO: 25 - DNA, 336 bp, Artificial Sequence
  Hu3A5(V3) VH nucleotide sequence
gatgtggtgatgacccagagtcccgacagcctggcggtgtctcttggggagcgggcgactattaactgcaaaagctcccagagcctagtccactcaaatggcaacacttacctgcactggtaccagcagaagcctggtcagccacccaagctgctcatctacaaggttagcaacaggttttcaggcgtccctgaccgcttcagtggctccggctccggcaccgacttcaccctgaccatctcttctttgcaggccgaggacgtggcggtttatttctgttctcaatccacccacgtccccttcaccttcggcggcgggaccaagctggagatcaaa

SEQ ID NO: 26 - DNA, 351 bp, Artificial Sequence
  Hu3A5(V3) VL nucleotide sequence
gaggtgcagctggtgcagtccggggcagaggtaaagaagccgggcgcttccgtgaaggtgtcgtgtaaggcttctggctacacgttcacatcctactggatgcattggatgcgccaggctcccggacagggcctggagtggatcggtgtgattgacccgagcgattcttacaccagctacaaccagaaatttcagggacgagtgactcttacggtggacacctcgacctccactgcctacatggagctgagctctctgcgctcggaagacaccgccgtgtactactgcgcccgtggtggcaagcgcgccatggattattggggccagggtaccacagtcaccgtgtcgtcc

SEQ ID NO: 27 - protein, 244 aa, Artificial Sequence
  Hu3A5(V3) scFv amino acid sequence
DVVMTQSPDSLAVSLGERATINCKSSQSLVHSNGNTYLHWYQQKPGQPPKLLIYKVSNRFSGVPDRFSGSGSGTDFTLTISSLQAEDVAVYFCSQSTHVPFTFGGGTKLEIKGGGGSGGGGSGGGGSEVQLVQSGAEVKKPGASVKVSCKASGYTFTSYWMHWMRQAPGQGLEWIGVIDPSDSYTSYNQKFQGRVTLTVDTSTSTAYMELSSLRSEDTAVYYCARGGKRAMDYWGQGTTVTVSS

SEQ ID NO: 28 - DNA, 732 bp, Artificial Sequence
  Hu3A5(V3) scFv nucleotide sequence
gatgtggtgatgacccagagtcccgacagcctggcggtgtctcttggggagcgggcgactattaactgcaaaagctcccagagcctagtccactcaaatggcaacacttacctgcactggtaccagcagaagcctggtcagccacccaagctgctcatctacaaggttagcaacaggttttcaggcgtccctgaccgcttcagtggctccggctccggcaccgacttcaccctgaccatctcttctttgcaggccgaggacgtggcggtttatttctgttctcaatccacccacgtccccttcaccttcggcggcgggaccaagctggagatcaaaggcggaggcggctccggtggggggggctcgggcggcggtggctccgaggtgcagctggtgcagtccggggcagaggtaaagaagccgggcgcttccgtgaaggtgtcgtgtaaggcttctggctacacgttcacatcctactggatgcattggatgcgccaggctcccggacagggcctggagtggatcggtgtgattgacccgagcgattcttacaccagctacaaccagaaatttcagggacgagtgactcttacggtggacacctcgacctccactgcctacatggagctgagctctctgcgctcggaagacaccgccgtgtactactgcgcccgtggtggcaagcgcgccatggattattggggccagggtaccacagtcaccgtgtcgtcc

SEQ ID NO: 29 - protein, 117 aa, Artificial Sequence; identical to SEQ ID NO: 11
  Hu3A5(V4) VH amino acid sequence

SEQ ID NO: 30 - protein, 112 aa, Artificial Sequence
  Hu3A5(V4) VL amino acid sequence
DVVMTQSPDSLAVSLGERATINCKSSQSLVHSNGNTYLHWYQQKPGQPPKLLIYKVSNRFSGVPDRFSGSGSGTDFTLTISSLQAEDVAVYYCSQSTHVPFTFGGGTKLEIK

SEQ ID NO: 31 - DNA, 336 bp, Artificial Sequence
  Hu3A5(V4) VH nucleotide sequence
gatgtggtgatgacccagtcccccgactcgctcgcggtgtccctgggcgagcgggctaccattaactgcaagtcctcccagtctttggtccactctaatggcaacacgtacctgcactggtaccagcagaagcccggccagccgcctaaactgcttatctacaaggtgtctaaccgcttctctggcgtcccagacaggttttcaggcagtgggtccggtaccgactttactctgaccatctcctcgctgcaggctgaggacgtggcggtatattactgttcgcagagcacacatgttcccttcaccttcggcgggggcaccaagttggagatcaag

SEQ ID NO: 32 - DNA, 351 bp, Artificial Sequence
  Hu3A5(V4) VL nucleotide sequence
gaggtgcagctggtgcaaagtggggcagaggtgaagaagcctggcgcttccgtgaaagtctcatgcaaggcctctggctacacgttcacctcttattggatgcactggatgcgccaggcccccggacagggactagagtggatcggtgtcattgacccgagcgatagctacacgagctacaaccagaaattccagggccgagtgactctcactgtggacacctcgacctccaccgcctacatggagctgagctccctgcgcagcgaagacacagcggtgtactactgtgcccgtgggggcaagcgcgccatggattattggggccagggtactaccgtgaccgtttcgagc

SEQ ID NO: 33 - protein, 244 aa, Artificial Sequence
  Hu3A5(V4) scFv amino acid sequence
DVVMTQSPDSLAVSLGERATINCKSSQSLVHSNGNTYLHWYQQKPGQPPKLLIYKVSNRFSGVPDRFSGSGSGTDFTLTISSLQAEDVAVYYCSQSTHVPFTFGGGTKLEIKGGGGSGGGGSGGGGSEVQLVQSGAEVKKPGASVKVSCKASGYTFTSYWMHWMRQAPGQGLEWIGVIDPSDSYTSYNQKFQGRVTLTVDTSTSTAYMELSSLRSEDTAVYYCARGGKRAMDYWGQGTTVTVSS

SEQ ID NO: 34 - DNA, 732 bp, Artificial Sequence
  Hu3A5(V4) scFv nucleotide sequence
gatgtggtgatgacccagtcccccgactcgctcgcggtgtccctgggcgagcgggctaccattaactgcaagtcctcccagtctttggtccactctaatggcaacacgtacctgcactggtaccagcagaagcccggccagccgcctaaactgcttatctacaaggtgtctaaccgcttctctggcgtcccagacaggttttcaggcagtgggtccggtaccgactttactctgaccatctcctcgctgcaggctgaggacgtggcggtatattactgttcgcagagcacacatgttcccttcaccttcggcgggggcaccaagttggagatcaagggtggcggaggttccggggggggcggctctggtggcggcggctccgaggtgcagctggtgcaaagtggggcagaggtgaagaagcctggcgcttccgtgaaagtctcatgcaaggcctctggctacacgttcacctcttattggatgcactggatgcgccaggcccccggacagggactagagtggatcggtgtcattgacccgagcgatagctacacgagctacaaccagaaattccagggccgagtgactctcactgtggacacctcgacctccaccgcctacatggagctgagctccctgcgcagcgaagacacagcggtgtactactgtgcccgtgggggcaagcgcgccatggattattggggccagggtactaccgtgaccgtttcgagc

SEQ ID NO: 35 - protein, 117 aa, Artificial Sequence
  Hu3A5(V5) VH amino acid sequence
QVQLVQSGAEVKKPGASVKVSCKASGYTFTSYWMHWVRQAPGQGLEWMGVIDPSDSYTSYNQKFQGRVTMTVDTSTSTAYMELSSLRSEDTAVYYCARGGKRAMDYWGQGTTVTVSS

SEQ ID NO: 36 - protein, 112 aa, Artificial Sequence; identical to SEQ ID NO: 12
  Hu3A5(V5) VL amino acid sequence

SEQ ID NO: 37 - DNA, 351 bp, Artificial Sequence
  Hu3A5(V5) VH nucleotide sequence
caggtccagctggtgcagagtggagcagaggtgaagaagcctggtgcgtctgttaaagtttcttgcaaggcgtccggctacacgttcacaagctattggatgcactgggtccgccaggccccagggcagggcttggagtggatgggcgtgattgacccgtccgacagctacaccagctacaaccagaaatttcagggacgtgtcactatgacagtggacacttcgacctctactgcctacatggaactttcctctctacgctcggaggacaccgccgtgtactactgtgctcgtgggggcaagcgcgccatggattattggggccagggcaccacggtcaccgtgtcctct

SEQ ID NO: 38 - DNA, 336 bp, Artificial Sequence
  Hu3A5(V5) VL nucleotide sequence
gacgtggtgatgacccagtcccccctgagccttccagtgaccctcggccagccggcttccatctcatgccgaagctcccagagcctcgtccactcaaatggcaacacgtacctgcactggttccagcagcggcccgggcagagccctcgcctgctgatctacaaggtgtcgaaccgcttctcgggcgtccccgacaggttttcgggttccggtagtggtaccgacttcaccctgaagatctcccgcgtggaggctgaggatgtgggcgtatacttttgttctcaatccactcatgtgcccttcaccttcggaggcggcaccaagctggagatcaag

SEQ ID NO: 39 - protein, 244 aa, Artificial Sequence
  Hu3A5(V5) scFv amino acid sequence
DVVMTQSPLSLPVTLGQPASISCRSSQSLVHSNGNTYLHWFQQRPGQSPRLLIYKVSNRFSGVPDRFSGSGSGTDFTLKISRVEAEDVGVYFCSQSTHVPFTFGGGTKLEIKGGGGSGGGGSGGGGSQVQLVQSGAEVKKPGASVKVSCKASGYTFTSYWMHWVRQAPGQGLEWMGVIDPSDSYTSYNQKFQGRVTMTVDTSTSTAYMELSSLRSEDTAVYYCARGGKRAMDYWGQGTTVTVSS

SEQ ID NO: 40 - DNA, 732 bp, Artificial Sequence
  Hu3A5(V5) scFv nucleotide sequence
gacgtggtgatgacccagtcccccctgagccttccagtgaccctcggccagccggcttccatctcatgccgaagctcccagagcctcgtccactcaaatggcaacacgtacctgcactggttccagcagcggcccgggcagagccctcgcctgctgatctacaaggtgtcgaaccgcttctcgggcgtccccgacaggttttcgggttccggtagtggtaccgacttcaccctgaagatctcccgcgtggaggctgaggatgtgggcgtatacttttgttctcaatccactcatgtgcccttcaccttcggaggcggcaccaagctggagatcaagggcgggggcgggtctggaggtggcggctccggtggtgggggctcccaggtccagctggtgcagagtggagcagaggtgaagaagcctggtgcgtctgttaaagtttcttgcaaggcgtccggctacacgttcacaagctattggatgcactgggtccgccaggccccagggcagggcttggagtggatgggcgtgattgacccgtccgacagctacaccagctacaaccagaaatttcagggacgtgtcactatgacagtggacacttcgacctctactgcctacatggaactttcctctctacgctcggaggacaccgccgtgtactactgtgctcgtgggggcaagcgcgccatggattattggggccagggcaccacggtcaccgtgtcctct

SEQ ID NO: 41 - protein, 117 aa, Artificial Sequence; identical to SEQ ID NO: 35
  Hu3A5(V6) VH amino acid sequence

SEQ ID NO: 42 - protein, 112 aa, Artificial Sequence; identical to SEQ ID NO: 18
  Hu3A5(V6) VL amino acid sequence

SEQ ID NO: 43 - DNA, 351 bp, Artificial Sequence
  Hu3A5(V6) VH nucleotide sequence
caggtgcagctagtgcagtctggggcggaggtgaagaagcctggcgcttccgtgaaagtttcgtgtaaggcatccggctacacgttcaccagctattggatgcattgggtccgccaggcccccggccagggtctggagtggatgggcgtgattgacccgtccgacagttacaccagttacaaccagaagttccagggccgggtgaccatgactgtggacacctcgacctccactgcctacatggagctgagcagcctgcgctcggaggacaccgcggtgtactactgcgcccgtggtgggaagcgcgccatggattattggggccagggcaccaccgtgactgtcagctcc

SEQ ID NO: 44 - DNA, 336 bp, Artificial Sequence
  Hu3A5(V6) VL nucleotide sequence
gatgtggtgatgacccagtcccctttgtcccttcccgtcaccttgggtcagccagcttctatctcttgccgaagctctcagtctctggtccactctaatggcaacacatacctgcactggttccagcagagaccaggtcagtcgccgcgcctgctgatctacaaggtgagcaaccgtttctccggagtccccgacaggttttcaggctccgggtcagggaccgactttacactcaaaatctcgcgcgtggaggctgaagatgttggcgtgtattactgttctcaaagcactcacgtacccttcaccttcggcggaggcaccaagctggagatcaag

SEQ ID NO: 45 - protein, 244 aa, Artificial Sequence
  Hu3A5(V6) scFv amino acid sequence
DVVMTQSPLSLPVTLGQPASISCRSSQSLVHSNGNTYLHWFQQRPGQSPRLLIYKVSNRFSGVPDRFSGSGSGTDFTLKISRVEAEDVGVYYCSQSTHVPFTFGGGTKLEIKGGGGSGGGGSGGGGSQVQLVQSGAEVKKPGASVKVSCKASGYTFTSYWMHWVRQAPGQGLEWMGVIDPSDSYTSYNQKFQGRVTMTVDTSTSTAYMELSSLRSEDTAVYYCARGGKRAMDYWGQGTTVTVSS

SEQ ID NO: 46 - DNA, 732 bp, Artificial Sequence
  Hu3A5(V6) scFv nucleotide sequence
gatgtggtgatgacccagtcccctttgtcccttcccgtcaccttgggtcagccagcttctatctcttgccgaagctctcagtctctggtccactctaatggcaacacatacctgcactggttccagcagagaccaggtcagtcgccgcgcctgctgatctacaaggtgagcaaccgtttctccggagtccccgacaggttttcaggctccgggtcagggaccgactttacactcaaaatctcgcgcgtggaggctgaagatgttggcgtgtattactgttctcaaagcactcacgtacccttcaccttcggcggaggcaccaagctggagatcaagggcgggggaggctccggtgggggcggtagcggcggcggaggctcccaggtgcagctagtgcagtctggggcggaggtgaagaagcctggcgcttccgtgaaagtttcgtgtaaggcatccggctacacgttcaccagctattggatgcattgggtccgccaggcccccggccagggtctggagtggatgggcgtgattgacccgtccgacagttacaccagttacaaccagaagttccagggccgggtgaccatgactgtggacacctcgacctccactgcctacatggagctgagcagcctgcgctcggaggacaccgcggtgtactactgcgcccgtggtgggaagcgcgccatggattattggggccagggcaccaccgtgactgtcagctcc

SEQ ID NO: 47 - protein, 117 aa, Artificial Sequence; identical to SEQ ID NO: 35
  Hu3A5(V7) VH amino acid sequence

SEQ ID NO: 48 - protein, 112 aa, Artificial Sequence; identical to SEQ ID NO: 24
  Hu3A5(V7) VL amino acid sequence

SEQ ID NO: 49 - DNA, 351 bp, Artificial Sequence
  Hu3A5(V7) VH nucleotide sequence
caagtgcagctggtgcagtccggcgcagaggtaaagaagcccggcgcttccgtgaaggtgtcctgtaaagcgtcgggctacacgttcaccagctattggatgcactgggtgcgccaggcccccgggcagggcctggagtggatgggcgtgattgacccgagtgacagctacaccagttacaaccagaaatttcagggacgtgtgaccatgactgtggacacctcgacctctactgcctacatggagctgtcctctctccgctcggaggacaccgccgtgtactactgcgcccgaggcggcaagcgcgccatggattattggggccagggcaccaccgtcaccgtgtcgtcc

SEQ ID NO: 50 - DNA, 336 bp, Artificial Sequence
  Hu3A5(V7) VL nucleotide sequence
gacgtggtgatgacccagagcccagattctctggcggtatctcttggcgagcgggctactatcaactgcaaatcttcccagagcctagtccacagcaatgggaacacgtacctgcattggtaccagcagaagcctggtcagccgcctaagctgctgatctacaaggttagcaaccgcttctccggtgtccccgacaggttttcaggctccggctccgggaccgacttcaccctgaccatctcgtctttgcaggctgaagatgtggcggtctacttctgttcacagagcacacacgttcccttcaccttcggcgggggcactaagctggagatcaag

SEQ ID NO: 51 - protein, 244 aa, Artificial Sequence
  Hu3A5(V7) scFv amino acid sequence
DVVMTQSPDSLAVSLGERATINCKSSQSLVHSNGNTYLHWYQQKPGQPPKLLIYKVSNRFSGVPDRFSGSGSGTDFTLTISSLQAEDVAVYFCSQSTHVPFTFGGGTKLEIKGGGGSGGGGSGGGGSQVQLVQSGAEVKKPGASVKVSCKASGYTFTSYWMHWVRQAPGQGLEWMGVIDPSDSYTSYNQKFQGRVTMTVDTSTSTAYMELSSLRSEDTAVYYCARGGKRAMDYWGQGTTVTVSS

SEQ ID NO: 52 - DNA, 732 bp, Artificial Sequence
  Hu3A5(V7) scFv nucleotide sequence
gacgtggtgatgacccagagcccagattctctggcggtatctcttggcgagcgggctactatcaactgcaaatcttcccagagcctagtccacagcaatgggaacacgtacctgcattggtaccagcagaagcctggtcagccgcctaagctgctgatctacaaggttagcaaccgcttctccggtgtccccgacaggttttcaggctccggctccgggaccgacttcaccctgaccatctcgtctttgcaggctgaagatgtggcggtctacttctgttcacagagcacacacgttcccttcaccttcggcgggggcactaagctggagatcaagggcggtggtggttccggcggaggaggctccggagggggtgggtctcaagtgcagctggtgcagtccggcgcagaggtaaagaagcccggcgcttccgtgaaggtgtcctgtaaagcgtcgggctacacgttcaccagctattggatgcactgggtgcgccaggcccccgggcagggcctggagtggatgggcgtgattgacccgagtgacagctacaccagttacaaccagaaatttcagggacgtgtgaccatgactgtggacacctcgacctctactgcctacatggagctgtcctctctccgctcggaggacaccgccgtgtactactgcgcccgaggcggcaagcgcgccatggattattggggccagggcaccaccgtcaccgtgtcgtcc

SEQ ID NO: 53 - protein, 117 aa, Artificial Sequence; identical to SEQ ID NO: 35
  Hu3A5(V8) VH amino acid sequence

SEQ ID NO: 54 - protein, 112 aa, Artificial Sequence; identical to SEQ ID NO: 30
  Hu3A5(V8) VL amino acid sequence

SEQ ID NO: 55 - DNA, 351 bp, Artificial Sequence
  Hu3A5(V8) VH nucleotide sequence
caggtccagctggtgcagtctggcgcggaggtgaagaagccaggtgcttccgtgaaagtgtcctgtaaggccagtggctacacgttcacaagctattggatgcactgggtgcgccaggcacccggacagggtctggaatggatgggcgtgattgacccgtccgacagttacaccagctacaaccagaaatttcagggacgtgtgaccatgacagttgacacctcgacttccactgcctacatggagctgtcctccctccgctcggaggacactgccgtgtactactgtgcccgaggcggcaagcgcgccatggattattggggccagggcacgaccgtcaccgtgtcgtca

SEQ ID NO: 56 - DNA, 336 bp, Artificial Sequence
  Hu3A5(V8) VL nucleotide sequence
gatgtggtgatgacccagagccctgactctttggcggtatcgctaggcgagcgggctaccatcaactgcaagtccagccagagccttgtccattctaatggcaacacgtacctgcactggtaccaacagaagcccgggcagccgcctaaactgctcatctacaaggtcagcaaccgcttctccggcgtccccgacaggttttcgggctccggctcagggaccgacttcaccctgaccatctcttctctgcaggccgaggatgtggcggtatactactgctctcagagcactcacgttcccttcaccttcggcggaggcaccaagctggagatcaag

SEQ ID NO: 57 - protein, 244 aa, Artificial Sequence
  Hu3A5(V8) scFv amino acid sequence
DVVMTQSPDSLAVSLGERATINCKSSQSLVHSNGNTYLHWYQQKPGQPPKLLIYKVSNRFSGVPDRFSGSGSGTDFTLTISSLQAEDVAVYYCSQSTHVPFTFGGGTKLEIKGGGGSGGGGSGGGGSQVQLVQSGAEVKKPGASVKVSCKASGYTFTSYWMHWVRQAPGQGLEWMGVIDPSDSYTSYNQKFQGRVTMTVDTSTSTAYMELSSLRSEDTAVYYCARGGKRAMDYWGQGTTVTVSS

SEQ ID NO: 58 - DNA, 732 bp, Artificial Sequence
  Hu3A5(V8) scFv nucleotide sequence
gatgtggtgatgacccagagccctgactctttggcggtatcgctaggcgagcgggctaccatcaactgcaagtccagccagagccttgtccattctaatggcaacacgtacctgcactggtaccaacagaagcccgggcagccgcctaaactgctcatctacaaggtcagcaaccgcttctccggcgtccccgacaggttttcgggctccggctcagggaccgacttcaccctgaccatctcttctctgcaggccgaggatgtggcggtatactactgctctcagagcactcacgttcccttcaccttcggcggaggcaccaagctggagatcaagggcgggggtgggtctgggggtggcggttccggaggtggaggctcccaggtccagctggtgcagtctggcgcggaggtgaagaagccaggtgcttccgtgaaagtgtcctgtaaggccagtggctacacgttcacaagctattggatgcactgggtgcgccaggcacccggacagggtctggaatggatgggcgtgattgacccgtccgacagttacaccagctacaaccagaaatttcagggacgtgtgaccatgacagttgacacctcgacttccactgcctacatggagctgtcctccctccgctcggaggacactgccgtgtactactgtgcccgaggcggcaagcgcgccatggattattggggccagggcacgaccgtcaccgtgtcgtca

SEQ ID NO: 59 - protein, 117 aa, Artificial Sequence
  Hu3A5(V9) VH amino acid sequence
EVQLVQSGSELKKPGASVKVSCKASGYTFTSYWMHWMRQAPGQGLEWIGVIDPSDSYTSYNQGFTGRFVLSVDTSVSTAYLQISSLKAEDTAVYYCARGGKRAMDYWGQGTTVTVSS

SEQ ID NO: 60 - protein, 112 aa, Artificial Sequence; identical to SEQ ID NO: 12
  Hu3A5(V9) VL amino acid sequence

SEQ ID NO: 61 - DNA, 351 bp, Artificial Sequence
  Hu3A5(V9) VH nucleotide sequence
gaggtgcagctggtgcagagcggttccgagctgaagaagcccggggcttccgtgaaggtgtcgtgtaaagcttctggctacacgttcacaagctattggatgcactggatgcgccaggcccctggtcagggactggagtggatcggcgtaattgacccgtccgacagctacactagctacaaccagggcttcaccggccgcttcgtcctttctgttgatacctccgtgtccactgcctacttgcaaatttcttctctgaaagcggaagacaccgccgtgtactactgcgctcgtggtggcaagcgcgccatggattattggggccagggcaccaccgtcaccgtgagcagc

SEQ ID NO: 62 - DNA, 336 bp, Artificial Sequence
  Hu3A5(V9) VL nucleotide sequence
gatgtggtgatgacccagtctcccctgagtctacctgtcactcttggacagccagcaagcatctcctgccgatcctcacagtccttggtacactcgaatggcaacacgtacctgcactggttccagcagagaccgggacagagcccacgcctgctcatctacaaggttagtaaccgcttttctggcgtccccgacaggttttcaggttccggcagtggaaccgactttactctgaagatctcccgggtggaggcggaggacgtgggcgtgtacttctgttcgcagtccacccatgtccccttcaccttcggcggcggcaccaagctggagatcaag

SEQ ID NO: 63 - protein, 244 aa, Artificial Sequence
  Hu3A5(V9) scFv amino acid sequence
DVVMTQSPLSLPVTLGQPASISCRSSQSLVHSNGNTYLHWFQQRPGQSPRLLIYKVSNRFSGVPDRFSGSGSGTDFTLKISRVEAEDVGVYFCSQSTHVPFTFGGGTKLEIKGGGGSGGGGSGGGGSEVQLVQSGSELKKPGASVKVSCKASGYTFTSYWMHWMRQAPGQGLEWIGVIDPSDSYTSYNQGFTGRFVLSVDTSVSTAYLQISSLKAEDTAVYYCARGGKRAMDYWGQGTTVTVSS

SEQ ID NO: 64 - DNA, 732 bp, Artificial Sequence
  Hu3A5(V9) scFv nucleotide sequence
gatgtggtgatgacccagtctcccctgagtctacctgtcactcttggacagccagcaagcatctcctgccgatcctcacagtccttggtacactcgaatggcaacacgtacctgcactggttccagcagagaccgggacagagcccacgcctgctcatctacaaggttagtaaccgcttttctggcgtccccgacaggttttcaggttccggcagtggaaccgactttactctgaagatctcccgggtggaggcggaggacgtgggcgtgtacttctgttcgcagtccacccatgtccccttcaccttcggcggcggcaccaagctggagatcaagggcggaggcggctcgggtggggggggctccggcgggggtgggtcggaggtgcagctggtgcagagcggttccgagctgaagaagcccggggcttccgtgaaggtgtcgtgtaaagcttctggctacacgttcacaagctattggatgcactggatgcgccaggcccctggtcagggactggagtggatcggcgtaattgacccgtccgacagctacactagctacaaccagggcttcaccggccgcttcgtcctttctgttgatacctccgtgtccactgcctacttgcaaatttcttctctgaaagcggaagacaccgccgtgtactactgcgctcgtggtggcaagcgcgccatggattattggggccagggcaccaccgtcaccgtgagcagc

SEQ ID NO: 65 - protein, 117 aa, Artificial Sequence; identical to SEQ ID NO: 59
  Hu3A5(V10) VH amino acid sequence

SEQ ID NO: 66 - protein, 112 aa, Artificial Sequence; identical to SEQ ID NO: 18
  Hu3A5(V10) VL amino acid sequence

SEQ ID NO: 67 - DNA, 351 bp, Artificial Sequence
  Hu3A5(V10) VH nucleotide sequence
gaggtgcagctggtgcagagcggttcggagctgaagaagccaggtgcatccgtgaaggtatcatgcaaagcttccggctacacgttcaccagctattggatgcattggatgcgccaggcccctgggcaggggcttgagtggatcggtgtgattgacccaagtgacagctacaccagctacaaccagggcttcaccggccggttcgtcctctccgttgataccagcgtatccacggcctacctgcaaatttccagcctgaaagcggaggacacagctgtttactactgtgctcgtggcgggaagcgcgccatggattattggggccagggcaccaccgtcaccgtgtcctct

SEQ ID NO: 68 - DNA, 336 bp, Artificial Sequence
  Hu3A5(V10) VL nucleotide sequence
gacgtggtgatgacccagagccccctgtcgctgccggtgactcttggacagccggcctccatctcttgccgatcttcccagtccttggtccactctaatggcaacacgtacttgcactggttccagcagcgtcccgggcagagccctcgcctgctgatctacaaggtgtcgaaccgcttctcgggcgtccccgacaggttttcaggctccggtagtggcaccgactttactctcaagatcagccgcgtggaggcggaagatgtgggcgtgtactactgttctcagtccactcacgtccccttcacctttggcggtgggaccaagctagagatcaag

SEQ ID NO: 69 - protein, 244 aa, Artificial Sequence
  Hu3A5(V10) scFv amino acid sequence
DVVMTQSPLSLPVTLGQPASISCRSSQSLVHSNGNTYLHWFQQRPGQSPRLLIYKVSNRFSGVPDRFSGSGSGTDFTLKISRVEAEDVGVYYCSQSTHVPFTFGGGTKLEIKGGGGSGGGGSGGGGSEVQLVQSGSELKKPGASVKVSCKASGYTFTSYWMHWMRQAPGQGLEWIGVIDPSDSYTSYNQGFTGRFVLSVDTSVSTAYLQISSLKAEDTAVYYCARGGKRAMDYWGQGTTVTVSS

SEQ ID NO: 70 - DNA, 732 bp, Artificial Sequence
  Hu3A5(V10) scFv nucleotide sequence
gacgtggtgatgacccagagccccctgtcgctgccggtgactcttggacagccggcctccatctcttgccgatcttcccagtccttggtccactctaatggcaacacgtacttgcactggttccagcagcgtcccgggcagagccctcgcctgctgatctacaaggtgtcgaaccgcttctcgggcgtccccgacaggttttcaggctccggtagtggcaccgactttactctcaagatcagccgcgtggaggcggaagatgtgggcgtgtactactgttctcagtccactcacgtccccttcacctttggcggtgggaccaagctagagatcaagggcggaggcgggtctggtggcggaggttctggagggggcggctccgaggtgcagctggtgcagagcggttcggagctgaagaagccaggtgcatccgtgaaggtatcatgcaaagcttccggctacacgttcaccagctattggatgcattggatgcgccaggcccctgggcaggggcttgagtggatcggtgtgattgacccaagtgacagctacaccagctacaaccagggcttcaccggccggttcgtcctctccgttgataccagcgtatccacggcctacctgcaaatttccagcctgaaagcggaggacacagctgtttactactgtgctcgtggcgggaagcgcgccatggattattggggccagggcaccaccgtcaccgtgtcctct

SEQ ID NO: 71 - protein, 117 aa, Artificial Sequence; identical to SEQ ID NO: 59
  Hu3A5(V11) VH amino acid sequence

SEQ ID NO: 72 - protein, 112 aa, Artificial Sequence; identical to SEQ ID NO: 24
  Hu3A5(V11) VL amino acid sequence

SEQ ID NO: 73 - DNA, 351 bp, Artificial Sequence
  Hu3A5(V11) VH nucleotide sequence
gaggtgcagctggtgcagagcggatcggagctgaagaagcccggggcttccgtgaaggtgtcgtgtaaggcttctggctacacgtttacaagctattggatgcattggatgcgccaggcgccgggtcagggtctggagtggatcggtgtgattgacccgagcgattcttacaccagctacaaccagggcttcaccggccgcttcgtcctgtccgtggacacctccgtgtccaccgcctacctgcaaatttcctctcttaaagcggaagacactgccgtgtactactgcgcccgcgggggcaagcgcgccatggattattggggccaggggactaccgtgactgtatcttcc

SEQ ID NO: 74 - DNA, 336 bp, Artificial Sequence
  Hu3A5(V11) VL nucleotide sequence
gatgtggtgatgacccagagtcccgacagcctagcagtttccctgggggagcgggctaccatcaactgcaaaagctcccagagccttgtccacagcaacggcaacacgtacttgcactggtaccagcagaagcctggacagccacccaaactgctcatctacaaggtttctaatcgtttttcaggcgtccctgacaggttttcaggctccggtagtggcaccgacttcaccctgaccatctcttctctgcaggccgaggacgtggcggtgtatttctgttcgcagtccacacacgtccccttcaccttcggcgggggcaccaagctggagatcaag

SEQ ID NO: 75 - protein, 244 aa, Artificial Sequence
  Hu3A5(V11) scFv amino acid sequence
DVVMTQSPDSLAVSLGERATINCKSSQSLVHSNGNTYLHWYQQKPGQPPKLLIYKVSNRFSGVPDRFSGSGSGTDFTLTISSLQAEDVAVYFCSQSTHVPFTFGGGTKLEIKGGGGSGGGGSGGGGSEVQLVQSGSELKKPGASVKVSCKASGYTFTSYWMHWMRQAPGQGLEWIGVIDPSDSYTSYNQGFTGRFVLSVDTSVSTAYLQISSLKAEDTAVYYCARGGKRAMDYWGQGTTVTVSS

SEQ ID NO: 76 - DNA, 732 bp, Artificial Sequence
  Hu3A5(V11) scFv nucleotide sequence
gatgtggtgatgacccagagtcccgacagcctagcagtttccctgggggagcgggctaccatcaactgcaaaagctcccagagccttgtccacagcaacggcaacacgtacttgcactggtaccagcagaagcctggacagccacccaaactgctcatctacaaggtttctaatcgtttttcaggcgtccctgacaggttttcaggctccggtagtggcaccgacttcaccctgaccatctcttctctgcaggccgaggacgtggcggtgtatttctgttcgcagtccacacacgtccccttcaccttcggcgggggcaccaagctggagatcaagggcggcggaggctccggagggggaggctcgggtggtggcggctccgaggtgcagctggtgcagagcggatcggagctgaagaagcccggggcttccgtgaaggtgtcgtgtaaggcttctggctacacgtttacaagctattggatgcattggatgcgccaggcgccgggtcagggtctggagtggatcggtgtgattgacccgagcgattcttacaccagctacaaccagggcttcaccggccgcttcgtcctgtccgtggacacctccgtgtccaccgcctacctgcaaatttcctctcttaaagcggaagacactgccgtgtactactgcgcccgcgggggcaagcgcgccatggattattggggccaggggactaccgtgactgtatcttcc

SEQ ID NO: 77 - protein, 117 aa, Artificial Sequence; identical to SEQ ID NO: 59
  Hu3A5(V12) VH amino acid sequence

SEQ ID NO: 78 - protein, 112 aa, Artificial Sequence; identical to SEQ ID NO: 30
  Hu3A5(V12) VL amino acid sequence

SEQ ID NO: 79 - DNA, 351 bp, Artificial Sequence
  Hu3A5(V12) VH nucleotide sequence
gaggtgcagctggtgcagagcggctcggagctgaagaagcccggggcttccgtgaaggtctcatgcaaagcgtctggctacacgttcactagctattggatgcactggatgcgccaggctcctgggcagggtctggagtggatcggtgtcattgacccgtccgacagttacaccagctacaaccagggcttcaccggccgcttcgtcttgtccgtagacacctccgtgtccaccgcctacctgcagatctcttctcttaaagcggaagatactgcagtgtactactgtgctcgtggtggcaagcgcgccatggattattggggccaggggaccacagtcaccgtgtcctcc

SEQ ID NO: 80 - DNA, 336 bp, Artificial Sequence
  Hu3A5(V12) VL nucleotide sequence
gatgtggtgatgacccagagcccggacagcctggccgtgtctctgggcgagcgggccactattaactgcaaatcctctcaatccctagtccactcaaatggcaacacgtacctccattggtaccagcagaagcctggacagccacccaagctgctgatctacaaggtgagcaaccgcttctctggtgttcccgacaggttttcaggctccggctcgggcaccgactttaccctgaccatctcgtccttgcaggccgaggacgtggcggtgtattactgttctcagagcactcacgttcccttcaccttcggcggaggcaccaagctggagatcaag

SEQ ID NO: 81 - protein, 244 aa, Artificial Sequence
  Hu3A5(V12) scFv amino acid sequence
DVVMTQSPDSLAVSLGERATINCKSSQSLVHSNGNTYLHWYQQKPGQPPKLLIYKVSNRFSGVPDRFSGSGSGTDFTLTISSLQAEDVAVYYCSQSTHVPFTFGGGTKLEIKGGGGSGGGGSGGGGSEVQLVQSGSELKKPGASVKVSCKASGYTFTSYWMHWMRQAPGQGLEWIGVIDPSDSYTSYNQGFTGRFVLSVDTSVSTAYLQISSLKAEDTAVYYCARGGKRAMDYWGQGTTVTVSS

SEQ ID NO: 82 - DNA, 732 bp, Artificial Sequence
  Hu3A5(V12) scFv nucleotide sequence
gatgtggtgatgacccagagcccggacagcctggccgtgtctctgggcgagcgggccactattaactgcaaatcctctcaatccctagtccactcaaatggcaacacgtacctccattggtaccagcagaagcctggacagccacccaagctgctgatctacaaggtgagcaaccgcttctctggtgttcccgacaggttttcaggctccggctcgggcaccgactttaccctgaccatctcgtccttgcaggccgaggacgtggcggtgtattactgttctcagagcactcacgttcccttcaccttcggcggaggcaccaagctggagatcaagggcgggggcggctccggtggtggaggtagtgggggagggggctccgaggtgcagctggtgcagagcggctcggagctgaagaagcccggggcttccgtgaaggtctcatgcaaagcgtctggctacacgttcactagctattggatgcactggatgcgccaggctcctgggcagggtctggagtggatcggtgtcattgacccgtccgacagttacaccagctacaaccagggcttcaccggccgcttcgtcttgtccgtagacacctccgtgtccaccgcctacctgcagatctcttctcttaaagcggaagatactgcagtgtactactgtgctcgtggtggcaagcgcgccatggattattggggccaggggaccacagtcaccgtgtcctcc

SEQ ID NO: 83 - protein, 117 aa, Artificial Sequence
  Hu3A5(V13) VH amino acid sequence
QVQLVQSGSELKKPGASVKVSCKASGYTFTSYWMNWVRQAPGQGLEWMGVIDPSDSYTSYNQGFTGRFVFSVDTSVSTAYLQISSLKAEDTAVYYCARGGKRAMDYWGQGTTVTVSS

SEQ ID NO: 84 - protein, 112 aa, Artificial Sequence; identical to SEQ ID NO: 12
  Hu3A5(V13) VL amino acid sequence

SEQ ID NO: 85 - DNA, 351 bp, Artificial Sequence
  Hu3A5(V13) VH nucleotide sequence
caggtgcagctggtgcagagcgggagcgagctgaagaagcccggggcttcggtgaaggtttcttgtaaggcgtccggctacacgttcactagctactggatgaactgggtccgccaggcccctggtcaggggctggagtggatgggcgtgattgacccgtccgactcctacacctcctacaaccagggcttcaccggccgcttcgtcttttctgtggacacctccgtttccaccgcctacctgcaaatttcctcgctgaaagcggaggacactgctgtatactactgtgcacgggggggcaaacgtgccatggattattggggccagggcacaaccgtgactgtctcctcc

SEQ ID NO: 86 - DNA, 336 bp, Artificial Sequence
  Hu3A5(V13) VL nucleotide sequence
gatgtggtgatgacccagagtccactctctctgcccgtgacccttggacagccggctagcatctcatgccgatcttcacagagcttggtgcattcaaatggcaacacttacctacactggttccagcagcgtccaggacagagccctcgcctgctgatctacaaggtgagcaaccgcttttccggtgtccccgacaggtttagtggttcgggctccggcaccgacttcaccttgaagatctctcgcgtggaggccgaagatgtgggggtgtatttctgctctcagagcacacacgtacccttcaccttcggcggcggcaccaagctggagatcaag

SEQ ID NO: 87 - protein, 244 aa, Artificial Sequence
  Hu3A5(V13) scFv amino acid sequence
DVVMTQSPLSLPVTLGQPASISCRSSQSLVHSNGNTYLHWFQQRPGQSPRLLIYKVSNRFSGVPDRFSGSGSGTDFTLKISRVEAEDVGVYFCSQSTHVPFTFGGGTKLEIKGGGGSGGGGSGGGGSQVQLVQSGSELKKPGASVKVSCKASGYTFTSYWMNWVRQAPGQGLEWMGVIDPSDSYTSYNQGFTGRFVFSVDTSVSTAYLQISSLKAEDTAVYYCARGGKRAMDYWGQGTTVTVSS

SEQ ID NO: 88 - DNA, 732 bp, Artificial Sequence
  Hu3A5(V13) scFv nucleotide sequence
gatgtggtgatgacccagagtccactctctctgcccgtgacccttggacagccggctagcatctcatgccgatcttcacagagcttggtgcattcaaatggcaacacttacctacactggttccagcagcgtccaggacagagccctcgcctgctgatctacaaggtgagcaaccgcttttccggtgtccccgacaggtttagtggttcgggctccggcaccgacttcaccttgaagatctctcgcgtggaggccgaagatgtgggggtgtatttctgctctcagagcacacacgtacccttcaccttcggcggcggcaccaagctggagatcaagggaggtggtgggtctggcggtggcggttcgggcggaggcggctcccaggtgcagctggtgcagagcgggagcgagctgaagaagcccggggcttcggtgaaggtttcttgtaaggcgtccggctacacgttcactagctactggatgaactgggtccgccaggcccctggtcaggggctggagtggatgggcgtgattgacccgtccgactcctacacctcctacaaccagggcttcaccggccgcttcgtcttttctgtggacacctccgtttccaccgcctacctgcaaatttcctcgctgaaagcggaggacactgctgtatactactgtgcacgggggggcaaacgtgccatggattattggggccagggcacaaccgtgactgtctcctcc

SEQ ID NO: 89 - protein, 117 aa, Artificial Sequence; identical to SEQ ID NO: 83
  Hu3A5(V14) VH amino acid sequence

SEQ ID NO: 90 - protein, 112 aa, Artificial Sequence; identical to SEQ ID NO: 18
  Hu3A5(V14) VL amino acid sequence

SEQ ID NO: 91 - DNA, 351 bp, Artificial Sequence
  Hu3A5(V14) VH nucleotide sequence
caggtccagctggtgcagtctgggtccgagctgaagaagcctggcgcgtccgtgaaggtgtcgtgtaaagcttccggctacaccttcaccagctattggatgaactgggtgcgccaggcccccgggcaggggctggagtggatgggcgtgattgacccgtccgattcttacacaagctacaaccagggcttcaccggccggttcgtgttctccgtggacacctccgttagcactgcctacctgcagatttcgtcgctcaaagcagaagacacggccgtgtactactgtgctcgcggcggcaagcgcgccatggattattggggccagggtacgaccgtcaccgtgtcctct

SEQ ID NO: 92 - DNA, 336 bp, Artificial Sequence
  Hu3A5(V14) VL nucleotide sequence
gatgtggtgatgacccagagccccctgtcccttccagtcaccctgggacagccagcttccatctcatgccgaagttctcagagtctagtccattctaatggcaacacttacctccactggttccagcagagacctgggcagtccccgcgcctgcttatctacaaggtcagcaaccgcttttcaggcgtacccgacaggttttcaggatcgggcagcgggaccgacttcacattgaagatctctcgtgtggaggcggaggacgtgggcgtgtactactgcagccaatcgactcacgttcccttcaccttcggcggaggcaccaagctggagatcaag

SEQ ID NO: 93 - protein, 244 aa, Artificial Sequence
  Hu3A5(V14) scFv amino acid sequence
DVVMTQSPLSLPVTLGQPASISCRSSQSLVHSNGNTYLHWFQQRPGQSPRLLIYKVSNRFSGVPDRFSGSGSGTDFTLKISRVEAEDVGVYYCSQSTHVPFTFGGGTKLEIKGGGGSGGGGSGGGGSQVQLVQSGSELKKPGASVKVSCKASGYTFTSYWMNWVRQAPGQGLEWMGVIDPSDSYTSYNQGFTGRFVFSVDTSVSTAYLQISSLKAEDTAVYYCARGGKRAMDYWGQGTTVTVSS

SEQ ID NO: 94 - DNA, 732 bp, Artificial Sequence
  Hu3A5(V14) scFv nucleotide sequence
gatgtggtgatgacccagagccccctgtcccttccagtcaccctgggacagccagcttccatctcatgccgaagttctcagagtctagtccattctaatggcaacacttacctccactggttccagcagagacctgggcagtccccgcgcctgcttatctacaaggtcagcaaccgcttttcaggcgtacccgacaggttttcaggatcgggcagcgggaccgacttcacattgaagatctctcgtgtggaggcggaggacgtgggcgtgtactactgcagccaatcgactcacgttcccttcaccttcggcggaggcaccaagctggagatcaagggcggcggcggttctgggggcggaggttccggtggtggtggttcccaggtccagctggtgcagtctgggtccgagctgaagaagcctggcgcgtccgtgaaggtgtcgtgtaaagcttccggctacaccttcaccagctattggatgaactgggtgcgccaggcccccgggcaggggctggagtggatgggcgtgattgacccgtccgattcttacacaagctacaaccagggcttcaccggccggttcgtgttctccgtggacacctccgttagcactgcctacctgcagatttcgtcgctcaaagcagaagacacggccgtgtactactgtgctcgcggcggcaagcgcgccatggattattggggccagggtacgaccgtcaccgtgtcctct

SEQ ID NO: 95 - protein, 117 aa, Artificial Sequence; identical to SEQ ID NO: 83
  Hu3A5(V15) VH amino acid sequence

SEQ ID NO: 96 - protein, 112 aa, Artificial Sequence; identical to SEQ ID NO: 24
  Hu3A5(V15) VL amino acid sequence

SEQ ID NO: 97 - DNA, 351 bp, Artificial Sequence
  Hu3A5(V15) VH nucleotide sequence
caggtgcagctggtgcagagcggcagcgagctgaagaagcctggggcttccgtaaaggtctcatgcaaggcttcgggctacacgttcacaagctattggatgaactgggtgcgccaggcccctggtcaggggctggagtggatgggcgtcattgacccgagtgacagctacaccagctacaaccagggcttcaccggccggttcgtcttttccgtggacacctccgtttccactgcctacctccaaatttcttctcttaaagccgaggacactgcagtgtactactgtgcgcgtggtggcaagcgcgccatggattactggggccagggtactaccgtcaccgtgtcgtcc

SEQ ID NO: 98 - DNA, 336 bp, Artificial Sequence
  Hu3A5(V15) VL nucleotide sequence
gatgtggtgatgacccagtcccccgattctctagccgtgtccctgggcgagcgcgctacaatcaactgcaaaagctcccagtccttggtgcacagcaatggcaacacgtacctgcattggtaccagcagaagcccggacagccaccgaagctgctcatctacaaggtgagcaaccgcttcagtggggtccccgacaggttttcaggctccggttcggggaccgactttactctgaccatctcctctctgcaggcggaagacgtggcggtatatttctgttctcagtccacccacgttcccttcaccttcggcggagggaccaagcttgagatcaaa

SEQ ID NO: 99 - protein, 244 aa, Artificial Sequence
  Hu3A5(V15) scFv amino acid sequence
DVVMTQSPDSLAVSLGERATINCKSSQSLVHSNGNTYLHWYQQKPGQPPKLLIYKVSNRFSGVPDRFSGSGSGTDFTLTISSLQAEDVAVYFCSQSTHVPFTFGGGTKLEIKGGGGSGGGGSGGGGSQVQLVQSGSELKKPGASVKVSCKASGYTFTSYWMNWVRQAPGQGLEWMGVIDPSDSYTSYNQGFTGRFVFSVDTSVSTAYLQISSLKAEDTAVYYCARGGKRAMDYWGQGTTVTVSS

SEQ ID NO: 100 - DNA, 732 bp, Artificial Sequence
  Hu3A5(V15) scFv nucleotide sequence
gatgtggtgatgacccagtcccccgattctctagccgtgtccctgggcgagcgcgctacaatcaactgcaaaagctcccagtccttggtgcacagcaatggcaacacgtacctgcattggtaccagcagaagcccggacagccaccgaagctgctcatctacaaggtgagcaaccgcttcagtggggtccccgacaggttttcaggctccggttcggggaccgactttactctgaccatctcctctctgcaggcggaagacgtggcggtatatttctgttctcagtccacccacgttcccttcaccttcggcggagggaccaagcttgagatcaaaggcggcggcggttctggaggtggtgggtctggcggcggaggctcccaggtgcagctggtgcagagcggcagcgagctgaagaagcctggggcttccgtaaaggtctcatgcaaggcttcgggctacacgttcacaagctattggatgaactgggtgcgccaggcccctggtcaggggctggagtggatgggcgtcattgacccgagtgacagctacaccagctacaaccagggcttcaccggccggttcgtcttttccgtggacacctccgtttccactgcctacctccaaatttcttctcttaaagccgaggacactgcagtgtactactgtgcgcgtggtggcaagcgcgccatggattactggggccagggtactaccgtcaccgtgtcgtcc

SEQ ID NO: 101 - protein, 117 aa, Artificial Sequence; identical to SEQ ID NO: 83
  Hu3A5(V16) VH amino acid sequence

SEQ ID NO: 102 - protein, 112 aa, Artificial Sequence; identical to SEQ ID NO: 30
  Hu3A5(V16) VL amino acid sequence

SEQ ID NO: 103 - DNA, 351 bp, Artificial Sequence
  Hu3A5(V16) VH nucleotide sequence
caggtgcagctggtgcagagcgggtccgagctcaagaagcccggcgcctcagtgaaggtatcgtgcaaggcttccggttacacgtttacctcttattggatgaactgggtccgccaggcccccggacaggggttggaatggatgggcgtcattgacccgtccgacagttacaccagctacaaccagggcttcactggccgtttcgtcttctccgtggacacttcggtctccaccgcttaccttcaaatttctagcctgaaagcggaggacaccgccgtgtattactgtgcacggggggggaagcgcgccatggattattggggccagggcacgaccgtcaccgtgagctct

SEQ ID NO: 104 - DNA, 336 bp, Artificial Sequence
  Hu3A5(V16) VL nucleotide sequence
gacgtggtgatgacccagtcgcccgattctttggccgtgtccctgggcgagcgcgcgaccatcaactgcaaatccagccagtccctagtgcactcaaatggcaacacgtacctgcactggtaccagcagaagcctggtcagccgcctaagctgctcatctacaaggtttcgaaccgcttctccggtgtgccagacaggttttctggttccggctccggaaccgacttcacactgaccatctcttccctgcaggcggaggatgtagccgtgtactactgttctcagtccacccatgtgccctttactttcggtgggggcactaaactggagatcaag

SEQ ID NO: 105 - protein, 244 aa, Artificial Sequence
  Hu3A5(V16) scFv amino acid sequence
DVVMTQSPDSLAVSLGERATINCKSSQSLVHSNGNTYLHWYQQKPGQPPKLLIYKVSNRFSGVPDRFSGSGSGTDFTLTISSLQAEDVAVYYCSQSTHVPFTFGGGTKLEIKGGGGSGGGGSGGGGSQVQLVQSGSELKKPGASVKVSCKASGYTFTSYWMNWVRQAPGQGLEWMGVIDPSDSYTSYNQGFTGRFVFSVDTSVSTAYLQISSLKAEDTAVYYCARGGKRAMDYWGQGTTVTVSS

SEQ ID NO: 106 - DNA, 732 bp, Artificial Sequence
  Hu3A5(V16) scFv nucleotide sequence
gacgtggtgatgacccagtcgcccgattctttggccgtgtccctgggcgagcgcgcgaccatcaactgcaaatccagccagtccctagtgcactcaaatggcaacacgtacctgcactggtaccagcagaagcctggtcagccgcctaagctgctcatctacaaggtttcgaaccgcttctccggtgtgccagacaggttttctggttccggctccggaaccgacttcacactgaccatctcttccctgcaggcggaggatgtagccgtgtactactgttctcagtccacccatgtgccctttactttcggtgggggcactaaactggagatcaagggcggaggcgggagcggcggcggcggaagtggcggaggtggcagccaggtgcagctggtgcagagcgggtccgagctcaagaagcccggcgcctcagtgaaggtatcgtgcaaggcttccggttacacgtttacctcttattggatgaactgggtccgccaggcccccggacaggggttggaatggatgggcgtcattgacccgtccgacagttacaccagctacaaccagggcttcactggccgtttcgtcttctccgtggacacttcggtctccaccgcttaccttcaaatttctagcctgaaagcggaggacaccgccgtgtattactgtgcacggggggggaagcgcgccatggattattggggccagggcacgaccgtcaccgtgagctct

SEQ ID NO: 107 - protein, 15 aa, Artificial Sequence
  linker amino acid sequence
GGGGSGGGGSGGGGS

SEQ ID NO: 108 - DNA, 45 bp, Artificial Sequence
  linker nucleotide sequence
ggcggcggaggctccggtggaggcgggtccgggggaggcggctcg

SEQ ID NO: 109 - DNA, 45 bp, Artificial Sequence
  linker nucleotide sequence
ggcgggggaggctccggcggaggcggctccggtggtggtggctcc

SEQ ID NO: 110 - DNA, 45 bp, Artificial Sequence
  linker nucleotide sequence
ggcggaggcggctccggtggggggggctcgggcggcggtggctcc

SEQ ID NO: 111 - DNA, 45 bp, Artificial Sequence
  linker nucleotide sequence
ggtggcggaggttccggggggggcggctctggtggcggcggctcc

SEQ ID NO: 112 - DNA, 45 bp, Artificial Sequence
  linker nucleotide sequence
ggcgggggcgggtctggaggtggcggctccggtggtgggggctcc

SEQ ID NO: 113 - DNA, 45 bp, Artificial Sequence
  linker nucleotide sequence
ggcgggggaggctccggtgggggcggtagcggcggcggaggctcc

SEQ ID NO: 114 - DNA, 45 bp, Artificial Sequence
  linker nucleotide sequence
ggcggtggtggttccggcggaggaggctccggagggggtgggtct

SEQ ID NO: 115 - DNA, 45 bp, Artificial Sequence
  linker nucleotide sequence
ggcgggggtgggtctgggggtggcggttccggaggtggaggctcc

SEQ ID NO: 116 - DNA, 45 bp, Artificial Sequence
  linker nucleotide sequence
ggcggaggcggctcgggtggggggggctccggcgggggtgggtcg

SEQ ID NO: 117 - DNA, 45 bp, Artificial Sequence
  linker nucleotide sequence
ggcggaggcgggtctggtggcggaggttctggagggggcggctcc

SEQ ID NO: 118 - DNA, 45 bp, Artificial Sequence
  linker nucleotide sequence
ggcggcggaggctccggagggggaggctcgggtggtggcggctcc

SEQ ID NO: 119 - DNA, 45 bp, Artificial Sequence
  linker nucleotide sequence
ggcgggggcggctccggtggtggaggtagtgggggagggggctcc

SEQ ID NO: 120 - DNA, 45 bp, Artificial Sequence
  linker nucleotide sequence
ggaggtggtgggtctggcggtggcggttcgggcggaggcggctcc

SEQ ID NO: 121 - DNA, 45 bp, Artificial Sequence
  linker nucleotide sequence
ggcggcggcggttctgggggcggaggttccggtggtggtggttcc

SEQ ID NO: 122 - DNA, 45 bp, Artificial Sequence
  linker nucleotide sequence
ggcggcggcggttctggaggtggtgggtctggcggcggaggctcc

SEQ ID NO: 123 - DNA, 45 bp, Artificial Sequence
  linker nucleotide sequence
ggcggaggcgggagcggcggcggcggaagtggcggaggtggcagc